European Patent Specification EP 4 049 674 B1, published April 29, 2026. Title: TRUNCATED EPIDERIMAL GROWTH FACTOR RECEPTOR (EGFRt) FOR TRANSDUCED T CELL SELECTION. Applicant: JENSEN, Michael C. Application PCT/US2010/055329. The sequence listing filed with the application follows.

SEQUENCE LISTING (6 sequences)

SEQ ID NO: 1 - DNA, 1071 bp, Homo sapiens
atgcttctcctggtgacaagccttctgctctgtgagttaccacacccagcattcctcctgatcccacgcaaagtgtgtaacggaataggtattggtgaatttaaagactcactctccataaatgctacgaatattaaacacttcaaaaactgcacctccatcagtggcgatctccacatcctgccggtggcatttaggggtgactccttcacacatactcctcctctggatccacaggaactggatattctgaaaaccgtaaaggaaatcacagggtttttgctgattcaggcttggcctgaaaacaggacggacctccatgcctttgagaacctagaaatcatacgcggcaggaccaagcaacatggtcagttttctcttgcagtcgtcagcctgaacataacatccttgggattacgctccctcaaggagataagtgatggagatgtgataatttcaggaaacaaaaatttgtgctatgcaaatacaataaactggaaaaaactgtttgggacctccggtcagaaaaccaaaattataagcaacagaggtgaaaacagctgcaaggccacaggccaggtctgccatgccttgtgctcccccgagggctgctggggcccggagcccagggactgcgtctcttgccggaatgtcagccgaggcagggaatgcgtggacaagtgcaaccttctggagggtgagccaagggagtttgtggagaactctgagtgcatacagtgccacccagagtgcctgcctcaggccatgaacatcacctgcacaggacggggaccagacaactgtatccagtgtgcccactacattgacggcccccactgcgtcaagacctgcccggcaggagtcatgggagaaaacaacaccctggtctggaagtacgcagacgccggccatgtgtgccacctgtgccatccaaactgcacctacggatgcactgggccaggtcttgaaggctgtccaacgaatgggcctaagatcccgtccatcgccactgggatggtgggggccctcctcttgctgctggtggtggccctggggatcggcctcttcatg

SEQ ID NO: 2 - DNA, 1071 bp, Homo sapiens
tacgaagaggaccactgttcggaagacgagacactcaatggtgtgggtcgtaaggaggactagggtgcgtttcacacattgccttatccataaccacttaaatttctgagtgagaggtatttacgatgcttataatttgtgaagtttttgacgtggaggtagtcaccgctagaggtgtaggacggccaccgtaaatccccactgaggaagtgtgtatgaggaggagacctaggtgtccttgacctataagacttttggcatttcctttagtgtcccaaaaacgactaagtccgaaccggacttttgtcctgcctggaggtacggaaactcttggatctttagtatgcgccgtcctggttcgttgtaccagtcaaaagagaacgtcagcagtcggacttgtattgtaggaaccctaatgcgagggagttcctctattcactacctctacactattaaagtcctttgtttttaaacacgatacgtttatgttatttgaccttttttgacaaaccctggaggccagtcttttggttttaatattcgttgtctccacttttgtcgacgttccggtgtccggtccagacggtacggaacacgagggggctcccgacgaccccgggcctcgggtccctgacgcagagaacggccttacagtcggctccgtcccttacgcacctgttcacgttggaagacctcccactcggttccctcaaacacctcttgagactcacgtatgtcacggtgggtctcacggacggagtccggtacttgtagtggacgtgtcctgcccctggtctgttgacataggtcacacgggtgatgtaactgccgggggtgacgcagttctggacgggccgtcctcagtaccctcttttgttgtgggaccagaccttcatgcgtctgcggccggtacacacggtggacacggtaggtttgacgtggatgcctacgtgacccggtccagaacttccgacaggttgcttacccggattctagggcaggtagcggtgaccctaccacccccgggaggagaacgacgaccaccaccgggacccctagccggagaagtac

SEQ ID NO: 3 - protein, 357 aa, Homo sapiens
MLLLVTSLLLCELPHPAFLLIPRKVCNGIGIGEFKDSLSINATNIKHFKNCTSISGDLHILPVAFRGDSFTHTPPLDPQELDILKTVKEITGFLLIQAWPENRTDLHAFENLEIIRGRTKQHGQFSLAVVSLNITSLGLRSLKEISDGDVIISGNKNLCYANTINWKKLFGTSGQKTKIISNRGENSCKATGQVCHALCSPEGCWGPEPRDCVSCRNVSRGRECVDKCNLLEGEPREFVENSECIQCHPECLPQAMNITCTGRGPDNCIQCAHYIDGPHCVKTCPAGVMGENNTLVWKYADAGHVCHLCHPNCTYGCTGPGLEGCPTNGPKIPSIATGMVGALLLLLVVALGIGLFM

SEQ ID NO: 4 - DNA, 3186 bp, Homo sapiens
atgctgctgctggtgaccagcctgctgctgtgcgagctgccccaccccgcctttctgctgatccccgacatccagatgacccagaccacctccagcctgagcgccagcctgggcgaccgggtgaccatcagctgccgggccagccaggacatcagcaagtacctgaactggtatcagcagaagcccgacggcaccgtcaagctgctgatctaccacaccagccggctgcacagcggcgtgcccagccggtttagcggcagcggctccggcaccgactacagcctgaccatctccaacctggaacaggaagatatcgccacctacttttgccagcagggcaacacactgccctacacctttggcggcggaacaaagctggaaatcaccggcagcacctccggcagcggcaagcctggcagcggcgagggcagcaccaagggcgaggtgaagctgcaggaaagcggccctggcctggtggcccccagccagagcctgagcgtgacctgcaccgtgagcggcgtgagcctgcccgactacggcgtgagctggatccggcagccccccaggaagggcctggaatggctgggcgtgatctggggcagcgagaccacctactacaacagcgccctgaagagccggctgaccatcatcaaggacaacagcaagagccaggtgttcctgaagatgaacagcctgcagaccgacgacaccgccatctactactgcgccaagcactactactacggcggcagctacgccatggactactggggccagggcaccagcgtgaccgtgagcagcgagagcaagtacggccctccctgccccccttgccctgcccccgagttcctgggcggacccagcgtgttcctgttcccccccaagcccaaggacaccctgatgatcagccggacccccgaggtgacctgcgtggtggtggacgtgagccaggaagatcccgaggtccagttcaattggtacgtggacggcgtggaagtgcacaacgccaagaccaagcccagagaggaacagttcaacagcacctaccgggtggtgtctgtgctgaccgtgctgcaccaggactggctgaacggcaaagaatacaagtgcaaggtgtccaacaagggcctgcccagcagcatcgaaaagaccatcagcaaggccaagggccagcctcgcgagccccaggtgtacaccctgcctccctcccaggaagagatgaccaagaaccaggtgtccctgacctgcctggtgaagggcttctaccccagcgacatcgccgtggagtgggagagcaacggccagcctgagaacaactacaagaccacccctcccgtgctggacagcgacggcagcttcttcctgtacagccggctgaccgtggacaagagccggtggcaggaaggcaacgtctttagctgcagcgtgatgcacgaggccctgcacaaccactacacccagaagagcctgagcctgtccctgggcaagatgttctgggtgctggtggtggtgggcggggtgctggcctgctacagcctgctggtgacagtggccttcatcatcttttgggtgcggagcaagcggagcagaggcggccacagcgactacatgaacatgacccccagacggcctggccccacccggaagcactaccagccctacgccccacccagggactttgccgcctaccggtccggcggagggcgggtgaagttcagcagaagcgccgacgcccctgcctaccagcagggccagaatcagctgtacaacgagctgaacctgggcagaagggaagagtacgacgtcctggataagcggagaggccgggaccctgagatgggcggcaagcctcggcggaagaacccccaggaaggcctgtataacgaactgcagaaagacaagatggccgaggcctacagcgagatcggcatgaagggcgagcggaggcggggcaagggccacgacggcctgtatcagggcctgtccaccgccaccaaggatacctacgacgccctgcacatgcaggccctgcccccaaggctcgagggcggcggagagggcagaggaagtcttctaacatgcggtgacgtggaggagaatcccggccctaggatgcttctcctggtgacaagccttctgctctgtgagttaccacacccagcattcctcctgatcccacgcaaagtgtgtaacggaataggtattggtgaatttaaagactcactctccataaatgctacgaatattaaacacttcaaaaactgcacctccatcagtggcgatctccacatcctgccggtggcatttaggggtgactccttcacacatactcctcctctggatccacaggaactggatattctgaaaaccgtaaaggaaatcacagggtttttgctgattcaggcttggcctgaaaacaggacggacctccatgcctttgagaacctagaaatcatacgcggcaggaccaagcaacatggtcagttttctcttgcagtcgtcagcctgaacataacatccttgggattacgctccctcaaggagataagtgatggagatgtgataatttcaggaaacaaaaatttgtgctatgcaaatacaataaactggaaaaaactgtttgggacctccggtcagaaaaccaaaattataagcaacagaggtgaaaacagctgcaaggccacaggccaggtctgccatgccttgtgctcccccgagggctgctggggcccggagcccagggactgcgtctcttgccggaatgtcagccgaggcagggaatgcgtggacaagtgcaaccttctggagggtgagccaagggagtttgtggagaactctgagtgcatacagtgccacccagagtgcctgcctcaggccatgaacatcacctgcacaggacggggaccagacaactgtatccagtgtgcccactacattgacggcccccactgcgtcaagacctgcccggcaggagtcatgggagaaaacaacaccctggtctggaagtacgcagacgccggccatgtgtgccacctgtgccatccaaactgcacctacggatgcactgggccaggtcttgaaggctgtccaacgaatgggcctaagatcccgtccatcgccactgggatggtgggggccctcctcttgctgctggtggtggccctggggatcggcctcttcatgtga

SEQ ID NO: 5 - DNA, 3186 bp, Homo sapiens
tacgacgacgaccactggtcggacgacgacacgctcgacggggtggggcggaaagacgactaggggctgtaggtctactgggtctggtggaggtcggactcgcggtcggacccgctggcccactggtagtcgacggcccggtcggtcctgtagtcgttcatggacttgaccatagtcgtcttcgggctgccgtggcagttcgacgactagatggtgtggtcggccgacgtgtcgccgcacgggtcggccaaatcgccgtcgccgaggccgtggctgatgtcggactggtagaggttggaccttgtccttctatagcggtggatgaaaacggtcgtcccgttgtgtgacgggatgtggaaaccgccgccttgtttcgacctttagtggccgtcgtggaggccgtcgccgttcggaccgtcgccgctcccgtcgtggttcccgctccacttcgacgtcctttcgccgggaccggaccaccgggggtcggtctcggactcgcactggacgtggcactcgccgcactcggacgggctgatgccgcactcgacctaggccgtcggggggtccttcccggaccttaccgacccgcactagaccccgtcgctctggtggatgatgttgtcgcgggacttctcggccgactggtagtagttcctgttgtcgttctcggtccacaaggacttctacttgtcggacgtctggctgctgtggcggtagatgatgacgcggttcgtgatgatgatgccgccgtcgatgcggtacctgatgaccccggtcccgtggtcgcactggcactcgtcgctctcgttcatgccgggagggacggggggaacgggacgggggctcaaggacccgcctgggtcgcacaaggacaagggggggttcgggttcctgtgggactactagtcggcctgggggctccactggacgcaccaccacctgcactcggtccttctagggctccaggtcaagttaaccatgcacctgccgcaccttcacgtgttgcggttctggttcgggtctctccttgtcaagttgtcgtggatggcccaccacagacacgactggcacgacgtggtcctgaccgacttgccgtttcttatgttcacgttccacaggttgttcccggacgggtcgtcgtagcttttctggtagtcgttccggttcccggtcggagcgctcggggtccacatgtgggacggagggagggtccttctctactggttcttggtccacagggactggacggaccacttcccgaagatggggtcgctgtagcggcacctcaccctctcgttgccggtcggactcttgttgatgttctggtggggagggcacgacctgtcgctgccgtcgaagaaggacatgtcggccgactggcacctgttctcggccaccgtccttccgttgcagaaatcgacgtcgcactacgtgctccgggacgtgttggtgatgtgggtcttctcggactcggacagggacccgttctacaagacccacgaccaccaccacccgccccacgaccggacgatgtcggacgaccactgtcaccggaagtagtagaaaacccacgcctcgttcgcctcgtctccgccggtgtcgctgatgtacttgtactgggggtctgccggaccggggtgggccttcgtgatggtcgggatgcggggtgggtccctgaaacggcggatggccaggccgcctcccgcccacttcaagtcgtcttcgcggctgcggggacggatggtcgtcccggtcttagtcgacatgttgctcgacttggacccgtcttcccttctcatgctgcaggacctattcgcctctccggccctgggactctacccgccgttcggagccgccttcttgggggtccttccggacatattgcttgacgtctttctgttctaccggctccggatgtcgctctagccgtacttcccgctcgcctccgccccgttcccggtgctgccggacatagtcccggacaggtggcggtggttcctatggatgctgcgggacgtgtacgtccgggacgggggttccgagctcccgccgcctctcccgtctccttcagaagattgtacgccactgcacctcctcttagggccgggatcctacgaagaggaccactgttcggaagacgagacactcaatggtgtgggtcgtaaggaggactagggtgcgtttcacacattgccttatccataaccacttaaatttctgagtgagaggtatttacgatgcttataatttgtgaagtttttgacgtggaggtagtcaccgctagaggtgtaggacggccaccgtaaatccccactgaggaagtgtgtatgaggaggagacctaggtgtccttgacctataagacttttggcatttcctttagtgtcccaaaaacgactaagtccgaaccggacttttgtcctgcctggaggtacggaaactcttggatctttagtatgcgccgtcctggttcgttgtaccagtcaaaagagaacgtcagcagtcggacttgtattgtaggaaccctaatgcgagggagttcctctattcactacctctacactattaaagtcctttgtttttaaacacgatacgtttatgttatttgaccttttttgacaaaccctggaggccagtcttttggttttaatattcgttgtctccacttttgtcgacgttccggtgtccggtccagacggtacggaacacgagggggctcccgacgaccccgggcctcgggtccctgacgcagagaacggccttacagtcggctccgtcccttacgcacctgttcacgttggaagacctcccactcggttccctcaaacacctcttgagactcacgtatgtcacggtgggtctcacggacggagtccggtacttgtagtggacgtgtcctgcccctggtctgttgacataggtcacacgggtgatgtaactgccgggggtgacgcagttctggacgggccgtcctcagtaccctcttttgttgtgggaccagaccttcatgcgtctgcggccggtacacacggtggacacggtaggtttgacgtggatgcctacgtgacccggtccagaacttccgacaggttgcttacccggattctagggcaggtagcggtgaccctaccacccccgggaggagaacgacgaccaccaccgggacccctagccggagaagtacact

SEQ ID NO: 6 - protein, 1061 aa, Homo sapiens [sequence omitted]